European Patent Application EP 4 610 271 A1, published September 3, 2025. Title: Self-assembling peptides and applications thereof. Applicant: Success Bio-Tech Co., Ltd. Application CN PCT/CN2023/098780, filed June 7, 2023. The sequence listing filed with the application follows.

SEQUENCE LISTING (6 sequences)

SEQ ID NO: 1 - protein, 13 aa, synthetic construct
PRVDVRVRVRVDP

SEQ ID NO: 2 - protein, 16 aa, synthetic construct
RADARADARADARADA

SEQ ID NO: 3 - protein, 9 aa, synthetic construct
PRVDVRVDP

SEQ ID NO: 4 - protein, 10 aa, synthetic construct
KLNLKLNLNL

SEQ ID NO: 5 - protein, 13 aa, synthetic construct
PRVDVRVKVRVDP

SEQ ID NO: 6 - protein, 10 aa, synthetic construct
RADMSRADMS